European Patent Application EP 4 438 035 A1, published October 2, 2024. Title: hGH 융합단백질의 고농도 투여 제형. Applicant: Genexine, Inc. The sequence listing filed with the application follows.

SEQUENCE LISTING (3 sequences)

SEQ ID NO: 1 - protein, 436 aa, synthetic construct
FPTIPLSRLFDNAMLRAHRLHQLAFDTYQEFEEAYIPKEQKYSFLQNPQTSLCFSESIPTPSNREETQQKSNLELLRISLLLIQSWLEPVQFLRSVFANSLVYGASDSNVYDLLKDLEEGIQTLMGRLEDGSPRTGQIFKQTYSKFDTNSHNDDALLKNYGLLYCFRKDMDKVETFLRIVQCRSVEGSCGFRNTGRGGEEKKKEKEKEEQEERETKTPECPSHTQPLGVFLFPPKPKDTLMISRTPEVTCVVVDVSQEDPEVQFNWYVDGVEVHNAKTKPREEQFNSTYRVVSVLTVLHQDWLNGKEYKCKVSNKGLPSSIEKTISKAKGQPREPQVYTLPPSQEEMTKNQVSLTCLVKGFYPSDIAVEWESNGQPENNYKTTPPVLDSDGSFFLYSRLTVDKSRWQEGNVFSCSVMHEALHNHYTQKSLSLSLGK

SEQ ID NO: 2 - protein, 191 aa, Homo sapiens [sequence omitted]

SEQ ID NO: 3 - protein, 245 aa, synthetic construct
RNTGRGGEEKKKEKEKEEQEERETKTPECPSHTQPLGVFLFPPKPKDTLMISRTPEVTCVVVDVSQEDPEVQFNWYVDGVEVHNAKTKPREEQFNSTYRVVSVLTVLHQDWLNGKEYKCKVSNKGLPSSIEKTISKAKGQPREPQVYTLPPSQEEMTKNQVSLTCLVKGFYPSDIAVEWESNGQPENNYKTTPPVLDSDGSFFLYSRLTVDKSRWQEGNVFSCSVMHEALHNHYTQKSLSLSLGK